European Patent Specification EP 3 375 875 B1, published April 15, 2026. Title: Separating Agent for Human IgG Polyclonal Antibody Derived from Serum and A Method for Separating the Antibody Using the Separating Agent. Applicant: National University Corporation Kyoto Institute of Technology Daicel Corporation. The sequence listing filed with the application follows.

SEQUENCE LISTING (147 sequences)

SEQ ID NO: 1 - DNA, 36 bp, Artificial Sequence
  primer
aaaaaggccatggcccagtcggtggaggagtccrgg

SEQ ID NO: 2 - DNA, 36 bp, Artificial Sequence
  primer
aaaaaggccatggcccagtcggtgaaggagtccgag

SEQ ID NO: 3 - DNA, 36 bp, Artificial Sequence
  primer
aaaaaggccatggcccagtcgytggaggagtccggg

SEQ ID NO: 4 - DNA, 38 bp, Artificial Sequence
  primer
aaaaaggccatggcccagsagcagctgrwggagtccgg

SEQ ID NO: 5 - DNA, 27 bp, Artificial Sequence
  primer
tccaccactagtgacggtgacsagggt

SEQ ID NO: 6 - DNA, 36 bp, Artificial Sequence
  primer
aattaaggatccgagctcgtgmtgacccagactsca

SEQ ID NO: 7 - DNA, 36 bp, Artificial Sequence
  primer
aattaaggatccgagctcgatmtgacccagactsca

SEQ ID NO: 8 - DNA, 36 bp, Artificial Sequence
  primer
aattaaggatccgagctcgtgatgacccagactgca

SEQ ID NO: 9 - DNA, 38 bp, Artificial Sequence
  primer
aattaaggatccgagctcgtgctgactcagtcgycctc

SEQ ID NO: 10 - DNA, 33 bp, Artificial Sequence
  primer
tatatatgcggccgccgaacstktgayswccac

SEQ ID NO: 11 - DNA, 35 bp, Artificial Sequence
  primer
tttaaatttgcggccgccgaacctgtgacggtcag

SEQ ID NO: 12 - protein, 121 aa, Oryctolagus cuniculus
QSVKESGGRLVTPGTPLTLTCTVSGIDLSSNAMSWVRQAPGEGLEWIGTISTVGKTYFASWAKGRFTISKTSTTVDLRITSPTTEDTATYFCATRYDSYGYAYNYWFGTLWGPGTLVTVTS

SEQ ID NO: 13 - protein, 117 aa, Oryctolagus cuniculus
QSVKESEGRLVTPGTPLTLTCTVSGFSLSRYAVSWVRQAPGKGLEWIGIIGSGGSTSYATWARGRFTISKTSTTVDLKITSPTTEDTVTYFCGSYYDSHGYAYVSLWGPGTLVTVTS

SEQ ID NO: 14 - protein, 119 aa, Oryctolagus cuniculus
QEQLVESGGGLVKPGGTLTLTCTVSGIDLSSYAMSWVRQVPGKGLEWIGIIGSGGGTAYANWAKGRFTISKTSSTTVDLKMTSLTTEDTATYFCATDYGIYGYAYGHLWGPGTLVTVTS

SEQ ID NO: 15 - protein, 118 aa, Oryctolagus cuniculus
QQQLMESGGRLVTPGGSLTLTCTVSGIDLNSYAMGWVRQAPGKGLEYIGIIRNSGNTYYASWAKGRFTISKTSSTTVDLKMTSLTTEDTATYFCARYSGDNGGALNLWGPGTLVTVTS

SEQ ID NO: 16 - protein, 121 aa, Oryctolagus cuniculus
QSLEESGGRLVTPGTPLTLTCTVSGIDLSSNAMTWVRQAPGEGLEWIGTISTGGSTYFASWAKGRFTISKTSTTVDLKITSPTTEDTATYFCATRYDSYGYAYNYWFGTLWGPGTLVTVTS

SEQ ID NO: 17 - protein, 116 aa, Oryctolagus cuniculus
QSVKESGGRLVTPGTPLTLTCTVSGFSLSSYAMGWVRQAPGKGLEYIGIISSSGSTYYASWAKGRFTISKTSTTVDLKITSPTTEDTATYFCARYSGDNGGALNLWGPGTLVTVTS

SEQ ID NO: 18 - protein, 116 aa, Oryctolagus cuniculus
QQQLMESGGGLVTPGTPLTLTCTVSGIDLRRYAMGWVRQAPGKGLQWIGIIASGNTDYASWAKGRFTISATSTTVDLKITSSTTEDTATYFCARYSGDNGGTLNLWGPGTLATVTT

SEQ ID NO: 19 - protein, 121 aa, Oryctolagus cuniculus; identical to SEQ ID NO: 16

SEQ ID NO: 20 - protein, 115 aa, Oryctolagus cuniculus
QSLEESGGRLVTPGTPLTLTCTVSGIDLRRYAMGWVRQAPGKGLQWIGIIASGNTDYASWAKGRFTISATSTTVDLKITSPTTEDTATYFCARYSGDNGGTLNLWGPGTLVTVTS

SEQ ID NO: 21 - protein, 112 aa, Oryctolagus cuniculus
ELDLTQTPPSVSGAVGGTVTIKCQASENINSELAWYQQKPGQRPKLLIYDASKLASGVPSRFSGSGSGTEYTLTISGMQCDDAATYYCQSTYYDGNYVYAFGGGTEVDVTRS

SEQ ID NO: 22 - protein, 111 aa, Oryctolagus cuniculus
ELVLTQTPSPVSGAVGGTVTINCQASQSISTALAWYQQKPGQPPKLLIYSASTLASGVSSRFKGSGSGTGFTLTISDLECADAATYYCQSYYGSSSDNAFGGGTEVVIKRS

SEQ ID NO: 23 - protein, 111 aa, Oryctolagus cuniculus
ELVMTQTASPVSAAVGGTVTIKCQASQSISTALAWYQQRPGQPPKLLIYDASTLASGVSSRFKGSGSGTEFTLTISDLECADAATYYCQTYFGSDTDNAFGEGTEVEITGS

SEQ ID NO: 24 - protein, 113 aa, Oryctolagus cuniculus
ELVMTQTAASVSGPVGGTVTIKCQASEFIRNYLAWYQQKPGQPPKLLIYTTSNLASGVPSRFSGSGSGTEYTLTISDLECADAATYYCQNYYDISTYGNAFGGGTEVVVIKGS

SEQ ID NO: 25 - protein, 112 aa, Oryctolagus cuniculus
ELVMTQTAASVSEPVGGTVTIKCQASQNINNELAWYQQKPGQRPKLLIYDASKLASGVPSRFSGSGSGTEFTLTISGMQCDDAATYYCQSTYYDGNYVYAFGGGTEVDVKGS

SEQ ID NO: 26 - protein, 112 aa, Oryctolagus cuniculus
ELDLTQTAASVSEPVGGTVTISCQSSQHIRSYLAWYQQKPGQPPKLLISAASTLASGVSSRFKGSGSGTEFTLTISDLECADAATYYCQRYYDIRNYGNGFGGGTEVEITGS

SEQ ID NO: 27 - protein, 112 aa, Oryctolagus cuniculus
ELVMTQTAASVSEPVGGTVTIKCQASEHIRNYLAWYQQKPGQPPKLLIYTTSNLASGVPSRFSGSGSGTEYTLTISDLECADAATYYCQNYYDISTYGNTFGGGTEVDVKGS

SEQ ID NO: 28 - protein, 112 aa, Oryctolagus cuniculus
ELVMTQTAASVSEPVGGTVTINCQASQSISDELAWYQQKPGQRPKLLIYDASDLASGVPSRFSGSGSGTEFTLTISGVQCDDAATYYCQSAYYDGRYVYAFGGGTEVEVTGS

SEQ ID NO: 29 - protein, 112 aa, Oryctolagus cuniculus
ELVMTQTAASVSEPVGGTVTIKCQASQSISSYLAWYQQKPGQPPKLLIYAASNLASGVSSRFKGSGSGTEFTLTISDLECADAATYYCQSYYSISSYGNTFGGGTEVEITGS

SEQ ID NO: 30 - protein, 19 aa, Oryctolagus cuniculus
ATRYDSYGYAYNYWFGTLW

SEQ ID NO: 31 - protein, 15 aa, Oryctolagus cuniculus
GSYYDSHGYAYVSLW

SEQ ID NO: 32 - protein, 15 aa, Oryctolagus cuniculus
ATDYGIYGYAYGHLW

SEQ ID NO: 33 - protein, 14 aa, Oryctolagus cuniculus
ARYSGDNGGTLNLW

SEQ ID NO: 34 - protein, 14 aa, Oryctolagus cuniculus
ARYSGDNGGALNLW

SEQ ID NO: 35 - protein, 8 aa, Artificial Sequence
  octapeptide
FVNQHLCK

SEQ ID NO: 36 - protein, 115 aa, Oryctolagus cuniculus
QSLEESGGRLVKPDETLTITCTASGFSLSSYAMGWVRQAPGKGLEWIGIIGSGDTYYASWAKGRFTISKTATTVDLKITSPTTEDTATYFCARAGNDRYIGDNLWGPGTLVTVTS

SEQ ID NO: 37 - protein, 114 aa, Oryctolagus cuniculus
SRWRSPGGRLVTPGTPLTITCTVSGIDLSSYAMIWVRQSPGEGLEYIGIISSTGSAYYASWAKGRFAIAKTSTTMDLKMTSPTTEDTATYFCGRYINGGYFDLWGPGTLVTVTS

SEQ ID NO: 38 - protein, 10 aa, Oryctolagus cuniculus
PRATLVTVTS

SEQ ID NO: 39 - protein, 114 aa, Oryctolagus cuniculus
QSLEESGGRLVTPGGSLTLTCTVSGIDLSSYAMGWVRQAPGKGLEWIGIVETGGSADYAAWAKGRFTISRTSTTVDLKITSPTTEDTATYFCVRDEHGNIGSLWGPGTLVTVTS

SEQ ID NO: 40 - protein, 10 aa, Oryctolagus cuniculus
PRATLVTVTS

SEQ ID NO: 41 - protein, 117 aa, Oryctolagus cuniculus
QSVEESRGRLVTPGTPLTLTCTVSGIDLNSWPMSWVRQAPGKGLEWIGIINTGGSAYYASWAEGRFTISKTSSTTVDLKITSPTTEDTATYFCARGVPSYGGGAYIWGPGTLVTVTS

SEQ ID NO: 42 - protein, 118 aa, Oryctolagus cuniculus
QQQLMESGGRLVTPGTPLTLTCTVSGIDLSGYAMGWVRQAPGKGLEYIGIIDATDVTYYASWAKGRFTISKASSTTVDLKLTSPTTEDTATYFCARYSGYNGGAFNLWGPGTLVTVTS

SEQ ID NO: 43 - protein, 10 aa, Oryctolagus cuniculus
PRATLVTVTS

SEQ ID NO: 44 - protein, 114 aa, Oryctolagus cuniculus
QSLEESGGRLVTPGTPLTLSCTVSGIDLSSNAMSWVRQAPGEGLEWIGAIYRGGNTEFASWANGRFTISKTSTTVDLKLTSLTTEDTATYFCAGDWDTLPFKFWGPGTLVTVTS

SEQ ID NO: 45 - protein, 122 aa, Oryctolagus cuniculus
QSVEESRGRLVTPGTPLTLTCTVSGFSLSTYGVSWVRQAPGKGLEYIGIISSSGSTYYANWAKGRFTISKTSSTTVDLKMTSLTTEDTATYFCARGGYSDSNYYIGYAFDPWGPGTLVTVTS

SEQ ID NO: 46 - protein, 115 aa, Oryctolagus cuniculus
QSVEESGGRLVSPGTPLTLTCTVSGFSLSSYYMIWVRQAPGKGLEYIGIIDGYGGSAYYASWAKGRFTFSRASTTVDLTMTSLTAADTATYFCARVDYGVSFDLWGPGTLVTVTS

SEQ ID NO: 47 - protein, 109 aa, Oryctolagus cuniculus
QSVKESRGRLVTPGTPLTLTCTASGFSLSSNAMSWVRQAPGEGLEWIGTINTGGTTYYASWAKGRFTISKTSTTVDLKMTGLTTEDTATYFCARFWNLWGPGTLVTVTS

SEQ ID NO: 48 - protein, 118 aa, Oryctolagus cuniculus
QEQLEESGGRLVTPGGSLTLTCTVSGIDLSSYAMGWVRQAPGKGLEYIGIISSSGSTYYASWARGRFTISKTSSTTVDLKMTSLTPEDTATYFCARYSGDNGGTLNLWGPGTLVTVTS

SEQ ID NO: 49 - protein, 117 aa, Oryctolagus cuniculus
QSLEESGGRLVTPGTPLTLTCTVSGLYLSSDAMIWVRQAPGKGLEWIGIIYASGSTYYASWAKGRFTISKTSTTVDLKITSPTTEDTATYFCAARVRSNGHYYFDLWGPGTLVTVTS

SEQ ID NO: 50 - protein, 116 aa, Oryctolagus cuniculus
QSVEESGGRLVTPGTPLTLTCTISGFSLNIYEINWVRQAPGKGLEWIAAIWREGHTDYSNWAKGRFTISKSSTTVELRMTSLTTEDTATYFCARYSGDNGGTFNLWGPGTLVTVTS

SEQ ID NO: 51 - protein, 116 aa, Oryctolagus cuniculus
QSLEESGGRLVTPGTPLTLTCTVSGFTISSYAMIWVRQAPGKGLEWIGAISSSGITYYASWAKGRFTISKTATTVDLKMTSLTTEDTATYFCARADYNTAAYFDLWGPGTLVTVTS

SEQ ID NO: 52 - protein, 19 aa, Oryctolagus cuniculus
ARGGYSDSNYYIGYAFDPW

SEQ ID NO: 53 - protein, 14 aa, Oryctolagus cuniculus
ARAGNDRYIGDNLW

SEQ ID NO: 54 - protein, 14 aa, Oryctolagus cuniculus
ARGVPSYGGGAYIW

SEQ ID NO: 55 - protein, 14 aa, Oryctolagus cuniculus
ARYSGYNGGAFNLW

SEQ ID NO: 56 - protein, 14 aa, Oryctolagus cuniculus
ARYSGDNGGTLNLW

SEQ ID NO: 57 - protein, 14 aa, Oryctolagus cuniculus
ARVRSNGHYYFDLW

SEQ ID NO: 58 - protein, 14 aa, Oryctolagus cuniculus
ARYSGDNGGTFNLW

SEQ ID NO: 59 - protein, 14 aa, Oryctolagus cuniculus
ARADYNTAAYFDLW

SEQ ID NO: 60 - protein, 12 aa, Oryctolagus cuniculus
GRYINGGYFDLW

SEQ ID NO: 61 - protein, 12 aa, Oryctolagus cuniculus
VRDEHGNIGSLW

SEQ ID NO: 62 - protein, 12 aa, Oryctolagus cuniculus
AGDWDTLPFKFW

SEQ ID NO: 63 - protein, 12 aa, Oryctolagus cuniculus
ARVDYGVSFDLW

SEQ ID NO: 64 - protein, 7 aa, Oryctolagus cuniculus
ARFWNLW

SEQ ID NO: 65 - protein, 122 aa, Oryctolagus cuniculus
QEQLMESGGRLVTPGTPLTLTCTVSGFSLSGYAVTWVRQAPGEGLEWIGTISTVGSTYFASWAKGRFTISKTSTTVDLKITSPTTEDTATYFCATRYDSYGYAYNYWFGTLWGPGTLVTVTS

SEQ ID NO: 66 - protein, 122 aa, Oryctolagus cuniculus
QQQLMESGGRLVTPGTPLTLTCTVSGIDLSSNAMTWVRQAPGEGLEWIGTISTGGSTYFASWAKGRFTISKTSTTVDLKITSPTTEDTATYFCATRYDSYGYAYNYWFGTLWGPGTLVTVTS

SEQ ID NO: 67 - protein, 117 aa, Oryctolagus cuniculus
QSVEESGGRLVSPGTPLTLTCTVSGFSLSSYYMIWVRQAPGKGLEYIGMIDGYGGNAYYANWAKGRFTVSKAATTVDLKMTSLTTEDTATYFCVRADYNTVSYFDLWGPGTLVTVTS

SEQ ID NO: 68 - protein, 121 aa, Oryctolagus cuniculus; identical to SEQ ID NO: 16

SEQ ID NO: 69 - protein, 121 aa, Oryctolagus cuniculus
QSLEESGGRLVTPGTPLTLTCTVSGIDLSDYAVTWVRQAPGKGLEWIGTISTYTNTYYASWAKGRFTISRTSTTVDLKITSPTTEDTATYFCATRYDSYGYAYNYWFGTLWGPGTLVTVTS

SEQ ID NO: 70 - protein, 122 aa, Oryctolagus cuniculus; identical to SEQ ID NO: 66

SEQ ID NO: 71 - protein, 115 aa, Oryctolagus cuniculus
QSLEESGGGLVTPGGSLTLACTVSGIDLSSNAMGWVRQAPGKGLEWIGLINSGGNTYYASWAKGRFTISRTSTTVDLQMTSPTTEDTATYFCARAGDSVSTLALWGPGTLVTVTS

SEQ ID NO: 72 - protein, 117 aa, Oryctolagus cuniculus
QSVEESGGRLVSPGTPLTLTCTASGFSLSTYYMIWVRQAPGKGLEYIGSIDGYDGDTYYATWAKGRFTVSKTATTVDLKMTSLTTEDTATYFCARADYNTVAYFDLWGPGTLVTVTS

SEQ ID NO: 73 - protein, 122 aa, Oryctolagus cuniculus; identical to SEQ ID NO: 66

SEQ ID NO: 74 - protein, 119 aa, Oryctolagus cuniculus
QSVEESRGRLVTPGTPLTLTCTVSGFSLSSYAMGWFRLAPGKGLEWIGIITIGDSIYYANWAKGRFTISKTSTTVDLRITSPTTADTATYFCARGNIGIGWGSYYFNFWGPGTLVTVTS

SEQ ID NO: 75 - protein, 115 aa, Oryctolagus cuniculus
QSVEESGGRLVTPGTPLTLTCTVSGIDLSSYAMSWVRQAPGKGLEWIGYITTRDKTYYTNWANGRFTISKTSTSVSLRIASPTTEDTATYFCATALYADDGNTLWGPGTLVTVTS

SEQ ID NO: 76 - protein, 114 aa, Oryctolagus cuniculus
QSLEESGGRLVTPGTPLTLTCTVSGFSLSSYPMGWFRQAPGKGLEYIGAINTGGSTYYASWARGRFTVSRTSTTVDLKMTSLTAEDTATYFCVRHDDDLTFNLWGPGTLVTVTS

SEQ ID NO: 77 - protein, 114 aa, Oryctolagus cuniculus
QQQLVESGGRLVTPGTPLTLTCTASGFSLSNYYMGWVRQAPGKGLQWIAYIMQSGTAYYASWARGRFTISRTSTTVDLKMPSLTAADTAAYFCARDVDGGYALWGPGTLVTVTS

SEQ ID NO: 78 - protein, 114 aa, Oryctolagus cuniculus
QSLEESGGRLVTPGTPLTLTCTASGFSLSSYYMSWVRQAPGKGLEWIGSIDTNSNTYYASWVKGRFTISKTSTTVDLKMTSPTTEDTATYFCVRGVIGATGDLWGPGTLVTVTS

SEQ ID NO: 79 - protein, 117 aa, Oryctolagus cuniculus
QSVEESRGRLVTPGTPLTLTCTVSGFSLSSYAISWVRQAPGKGLEWIGYILAGGSAYYANWAKGRFTISKTSTTVELKVTSPTTEDTATYFCARGGAGYNTVGLNLWGPGTLVTVTS

SEQ ID NO: 80 - protein, 122 aa, Oryctolagus cuniculus; identical to SEQ ID NO: 65

SEQ ID NO: 81 - protein, 117 aa, Oryctolagus cuniculus; identical to SEQ ID NO: 67

SEQ ID NO: 82 - protein, 115 aa, Oryctolagus cuniculus
QSVKESEGRLVTPGTPLTLTCTVSGFSLSNYNMQWVRQAPGKGLEYIGAIYSSGPTYYASWAKGRFTISKTSTTVDLEMTSLTSEDTATYFCAKNDDPFETYDLWGPGTLVTVTS

SEQ ID NO: 83 - protein, 116 aa, Oryctolagus cuniculus
QSVEESRGRLVTPGTPLTLTCTVSGIDLMSNAMGWVRQAPGKGLEYIGIISSSGSTYYASWAKGRFTISKTSTTVDLKITSPTTEDAATYFCARAIGDNGGYFNLWGPGTLVTVTS

SEQ ID NO: 84 - protein, 114 aa, Oryctolagus cuniculus
QEQLEESGGGLVTPGTPLTLTCTASGFSLDSYYMIWVRQAPGEGLEWIGIIGGGGDTAYASWAKGRFTISKTSTTVDLKMTSLTTEDTATYFCARDVDGGYALWGPGTLVTVTS

SEQ ID NO: 85 - protein, 121 aa, Oryctolagus cuniculus; identical to SEQ ID NO: 16

SEQ ID NO: 86 - protein, 119 aa, Oryctolagus cuniculus
QSVEESGGRLVTPGTPLTLTCTVSGIDLNNYAMGWVRQAPGKGLEYIGIISYGGSAYYASWAKGRFTISRTSTTVDLKITSPTTEDTATYFCARGDYDNYGYGYAINFWGPGTLVTVTS

SEQ ID NO: 87 - protein, 112 aa, Oryctolagus cuniculus
QSVEESGGRLVTPGTPLTLTCTVSGIDLSSYPMGWVRQAPGKGLEYIGIISDSDNTYYASWAKGRFTISKTSTTVDLKITSPTTEDTATYFCARGWLYFDLWGPGTLVTVTS

SEQ ID NO: 88 - protein, 117 aa, Oryctolagus cuniculus
QSLEESGGRLVTPGTPLTLTCTVSGIDLNSYAMGWVRQAPGEGLEWIGIITSSSITYYASWAKGRFTISKTSTTVDLKMTSLTTEDTATYFCARGDYNNNWDYFNLWGPGTLVTVTS

SEQ ID NO: 89 - protein, 116 aa, Oryctolagus cuniculus; identical to SEQ ID NO: 50

SEQ ID NO: 90 - protein, 118 aa, Oryctolagus cuniculus
QSLEESGGRLVTPGTPLTLTCTVSGFSLSSYAMNWVRQAPGKGLEWITFIGTGGDIYYANWAKGRFTISKTSTTVDLKIASPTTEDTATYFCARGDTGGSLYRHFNLWGPGTLVTVTS

SEQ ID NO: 91 - protein, 19 aa, Oryctolagus cuniculus
ATRYDSYGYAYNYWFGTLW

SEQ ID NO: 92 - protein, 17 aa, Oryctolagus cuniculus
ARGNIGIGWGSYYFNFW

SEQ ID NO: 93 - protein, 17 aa, Oryctolagus cuniculus
ARGDYDNYGYGYAINFW

SEQ ID NO: 94 - protein, 16 aa, Oryctolagus cuniculus
ARGDTGGSLYRHFNLW

SEQ ID NO: 95 - protein, 15 aa, Oryctolagus cuniculus
ARGGAGYNTVGLNLW

SEQ ID NO: 96 - protein, 15 aa, Oryctolagus cuniculus
ARGDYNNNWDYFNLW

SEQ ID NO: 97 - protein, 14 aa, Oryctolagus cuniculus
ARADYNTVAYFDLW

SEQ ID NO: 98 - protein, 14 aa, Oryctolagus cuniculus
VRADYNTVSYFDLW

SEQ ID NO: 99 - protein, 14 aa, Oryctolagus cuniculus
ARAIGDNGGYFNLW

SEQ ID NO: 100 - protein, 14 aa, Oryctolagus cuniculus
ARYSGDNGGTFNLW

SEQ ID NO: 101 - protein, 13 aa, Oryctolagus cuniculus
ARAGDSVSTLALW

SEQ ID NO: 102 - protein, 13 aa, Oryctolagus cuniculus
ATALYADDGNTLW

SEQ ID NO: 103 - protein, 13 aa, Oryctolagus cuniculus
AKNDDPFETYDLW

SEQ ID NO: 104 - protein, 12 aa, Oryctolagus cuniculus
VRGVIGATGDLW

SEQ ID NO: 105 - protein, 12 aa, Oryctolagus cuniculus
VRHDDDLTFNLW

SEQ ID NO: 106 - protein, 11 aa, Oryctolagus cuniculus
ARDVDGGYALW

SEQ ID NO: 107 - protein, 10 aa, Oryctolagus cuniculus
ARGWLYFDLW

SEQ ID NO: 108 - protein, 121 aa, Oryctolagus cuniculus; identical to SEQ ID NO: 12

SEQ ID NO: 109 - protein, 122 aa, Oryctolagus cuniculus; identical to SEQ ID NO: 66

SEQ ID NO: 110 - protein, 112 aa, Oryctolagus cuniculus
QSLEESGGRLVTPGGSLTLTCTASGFSLSAYDINWVRQAPGKGLEWIGMISGSGSTYYASWAKGRFTISKTSTTVDLKMTSLTAADTATYFCARGFDNYNLWGPGTLVTVTS

SEQ ID NO: 111 - protein, 122 aa, Oryctolagus cuniculus; identical to SEQ ID NO: 66

SEQ ID NO: 112 - protein, 121 aa, Oryctolagus cuniculus
QSVEESGGRLVTPGTPLTLTCTVSGIDLSSNAMTWVRQAPGEGLEWIGTISTGGSTYFASWAKGRFTISKTSTTVDLKITSPTTEDTATYFCATRYDSYGYAYNYWFGTLWGPGTLVTVTS

SEQ ID NO: 113 - protein, 121 aa, Oryctolagus cuniculus; identical to SEQ ID NO: 16

SEQ ID NO: 114 - protein, 121 aa, Oryctolagus cuniculus
QSLEESGGRLVTPGTPLTLTCTVSGIDLSNNAMSWVRQAPGEGLEWIGTISTGGSAYYASWAKGRFTISKTSTTVDLKITSPTTEDTATYFCATRYDSYGYAYNYWFGTLWGPGTLVTVTS

SEQ ID NO: 115 - protein, 122 aa, Oryctolagus cuniculus; identical to SEQ ID NO: 66

SEQ ID NO: 116 - protein, 121 aa, Oryctolagus cuniculus; identical to SEQ ID NO: 12

SEQ ID NO: 117 - protein, 121 aa, Oryctolagus cuniculus; identical to SEQ ID NO: 16

SEQ ID NO: 118 - protein, 121 aa, Oryctolagus cuniculus; identical to SEQ ID NO: 16

SEQ ID NO: 119 - protein, 122 aa, Oryctolagus cuniculus; identical to SEQ ID NO: 66

SEQ ID NO: 120 - protein, 117 aa, Oryctolagus cuniculus; identical to SEQ ID NO: 67

SEQ ID NO: 121 - protein, 121 aa, Oryctolagus cuniculus; identical to SEQ ID NO: 16

SEQ ID NO: 122 - protein, 121 aa, Oryctolagus cuniculus; identical to SEQ ID NO: 16

SEQ ID NO: 123 - protein, 121 aa, Oryctolagus cuniculus; identical to SEQ ID NO: 16

SEQ ID NO: 124 - protein, 122 aa, Oryctolagus cuniculus; identical to SEQ ID NO: 66

SEQ ID NO: 125 - protein, 121 aa, Oryctolagus cuniculus; identical to SEQ ID NO: 112

SEQ ID NO: 126 - protein, 117 aa, Oryctolagus cuniculus; identical to SEQ ID NO: 72

SEQ ID NO: 127 - protein, 121 aa, Oryctolagus cuniculus; identical to SEQ ID NO: 16

SEQ ID NO: 128 - protein, 121 aa, Oryctolagus cuniculus; identical to SEQ ID NO: 16

SEQ ID NO: 129 - protein, 122 aa, Oryctolagus cuniculus; identical to SEQ ID NO: 66

SEQ ID NO: 130 - protein, 122 aa, Oryctolagus cuniculus; identical to SEQ ID NO: 66

SEQ ID NO: 131 - protein, 121 aa, Oryctolagus cuniculus; identical to SEQ ID NO: 114

SEQ ID NO: 132 - protein, 122 aa, Oryctolagus cuniculus; identical to SEQ ID NO: 66

SEQ ID NO: 133 - protein, 117 aa, Oryctolagus cuniculus
QSVKESGGRLVSPGTPLTLTCTVSGFSLSSYYMIWVRQAPGKGLEYIGSIDGYDGDTYYATWAKGRFTVSKTATTVDLKMTSLTTEDTATYFCARADYNTVAYFDLWGPGTLVTVTS

SEQ ID NO: 134 - protein, 121 aa, Oryctolagus cuniculus; identical to SEQ ID NO: 16

SEQ ID NO: 135 - protein, 121 aa, Oryctolagus cuniculus
QSLEESGGRLVTPGTPLTLTCTVSGIDLSSNAMTWVRQAPGEGLEWIGTISTIGTTYFASWAKGRFTISKTSTTVDLKITSPTTEDTATYFCATRYDSYGYAYNYWFGTLWGPGTLVTVTS

SEQ ID NO: 136 - protein, 117 aa, Oryctolagus cuniculus
QSLEESGGRLVSPGTPLTLTCTVSGFSLSTYYMIWVRQAPGKGLEYIGSIDGYGGNAYYATWAKGRFTISKTATTVDLKMTSLTTEDTATYFCARADYNTAAYFDLWGPGTLVTVTS

SEQ ID NO: 137 - protein, 121 aa, Oryctolagus cuniculus; identical to SEQ ID NO: 16

SEQ ID NO: 138 - protein, 121 aa, Oryctolagus cuniculus; identical to SEQ ID NO: 16

SEQ ID NO: 139 - protein, 117 aa, Oryctolagus cuniculus
QSLEESGGRLVTPGTPLTLTCTVSGFSLSSYYMIWVRQAPGKGLEYIGSIDGYGGSAYYATWAKGRFTVSKTATTVDLKMTSLTTEDTATYFCARADYNTAAYFDLWGPGTLVTVTS

SEQ ID NO: 140 - protein, 19 aa, Oryctolagus cuniculus
ATRYDSYGYAYNYWFGTLW

SEQ ID NO: 141 - protein, 14 aa, Oryctolagus cuniculus
ARADYNTVAYFDLW

SEQ ID NO: 142 - protein, 14 aa, Oryctolagus cuniculus
ARADYNTAAYFDLW

SEQ ID NO: 143 - protein, 14 aa, Oryctolagus cuniculus
VRADYNTVSYFDLW

SEQ ID NO: 144 - protein, 10 aa, Oryctolagus cuniculus
ARGFDNYNLW

SEQ ID NO: 145 - protein, 121 aa, Oryctolagus cuniculus; identical to SEQ ID NO: 112

SEQ ID NO: 146 - protein, 121 aa, Oryctolagus cuniculus; identical to SEQ ID NO: 112

SEQ ID NO: 147 - protein, 121 aa, Oryctolagus cuniculus; identical to SEQ ID NO: 12